European Patent Specification EP 3 917 957 B1, published November 26, 2025. Title: PSMP Antagonsits for Use in Treatment of Disease. Applicant: Maple Biotech LLC. The sequence listing filed with the application follows.

SEQUENCE LISTING (7 sequences)

SEQ ID NO: 1 - protein, 139 aa, Homo sapiens
  SIGNAL (1)..(36)
MALRMLWAGQAKGILGGWGIICLVMSLLLQHPGVYSKCYFQAQAPCHYEGKYFTLGESWLRKDCFHCTCLHPVGVGCCDTSQHPIDFPAGCEVRQEAGTCQFSLVQKSDPRLPCKGGGPDPEWGSANTPVPGAPAPHSS

SEQ ID NO: 2 - protein, 374 aa, Homo sapiens
MLSTSRSRFIRNTNESGEEVTTFFDYDYGAPCHKFDVKQIGAQLLPPLYSLVFIFGFVGNMLVVLILINCKKLKCLTDIYLLNLAISDLLFLITLPLWAHSAANEWVFGNAMCKLFTGLYHIGYFGGIFFIILLTIDRYLAIVHAVFALKARTVTFGVVTSVITWLVAVFASVPGIIFTKCQKEDSVYVCGPYFPRGWNNFHTIMRNILGLVLPLLIMVICYSGILKTLLRCRNEKKRHRAVRVIFTIMIVYFLFWTPYNIVILLNTFQEFFGLSNCESTSQLDQATQVTETLGMTHCCINPIIYAFVGEKFRSLFHIALGCRIAPLQKPVCGGPGVRPGKNVKVTTQGLLDGRGKGKSIGRAPEASLQDKEGA

SEQ ID NO: 3 - protein, 360 aa, Homo sapiens
MLSTSRSRFIRNTNESGEEVTTFFDYDYGAPCHKFDVKQIGAQLLPPLYSLVFIFGFVGNMLVVLILINCKKLKCLTDIYLLNLAISDLLFLITLPLWAHSAANEWVFGNAMCKLFTGLYHIGYFGGIFFIILLTIDRYLAIVHAVFALKARTVTFGVVTSVITWLVAVFASVPGIIFTKCQKEDSVYVCGPYFPRGWNNFHTIMRNILGLVLPLLIMVICYSGILKTLLRCRNEKKRHRAVRVIFTIMIVYFLFWTPYNIVILLNTFQEFFGLSNCESTSQLDQATQVTETLGMTHCCINPIIYAFVGEKFRRYLSVFFRKHITKRFCKQCPVFYRETVDGVTSTNTPSTGEQEVSAGL

SEQ ID NO: 4 - protein, 119 aa, Mus musculus
EVQLQQSGPELVKPGASVKISCKASGYSFTGYFMNWVMQSHGKSLEWIGRINPYNGDTFYNQKFKGKATLTVDKSSSTAHMELRSLASEDSAVYYCARGGDGYYAFAYWGQGTLVTVSA

SEQ ID NO: 5 - protein, 108 aa, Mus musculus
NIVMTQSPKSMSMSVGERVTLSCRASENVGTYVSWYQQKPEQSPKLLIYGASNRYTGVPDRFTGSGSATDFTLTISSVQAEDLADYHCGQSYSYMYTFGGGTKLEIKR

SEQ ID NO: 6 - DNA, 357 bp, Mus musculus
gaggttcagctgcagcagtctggacctgagctggtgaagcctggggcttcagtgaagatatcctgcaaggcttctggttactcatttactggctactttatgaactgggtgatgcagagccatggaaagagccttgagtggattggacgtattaatccttacaatggtgatactttctacaaccagaagttcaagggcaaggccacattgactgtagacaaatcctctagtacagcccacatggagctccggagcctggcatctgaggactctgcagtctattattgtgcaagaggtggggatggttactacgcgtttgcttactggggccaagggactctggtcactgtctctgca

SEQ ID NO: 7 - DNA, 324 bp, Mus musculus
aacattgtaatgacccaatctcccaaatccatgtccatgtcagtaggagagagggtcaccttgagctgcagggccagtgagaatgtgggtacttatgtatcctggtatcaacagaaaccagagcagtctcctaaactgctgatatacggggcatccaaccggtacactggggtccccgatcgcttcacaggcagtggatctgcaacagatttcactctgaccatcagcagtgtgcaggctgaagaccttgcagattatcactgtggacagagttacagctatatgtacacgttcggaggggggaccaagctggaaataaaacgg